European Patent Specification EP 4 441 079 B1, published February 11, 2026. Title: Switchable polypeptide and its use for gentle affinity purification. Applicant: OXFORD UNIVERSITY INNOVATION LIMITED. Application WO. The sequence listing filed with the application follows.

SEQUENCE LISTING (19 sequences)

SEQ ID NO: 1 - protein, 113 aa, synthetic construct
  VARIANT 77: note = wherein X is selected from A, G, S, N or T
  source 1..113: note = SpySwitch variant
VTTLSGLSGEQGPSGDMTTEEDSATHIHFHKHDEDGRELAGATMELRDCSGKTISTWITDGHVKDFYLYPGKYTFVXTAAPDGHHVATPIEFTINEDGQVTVDGEATEGDPHT

SEQ ID NO: 2 - protein, 92 aa, synthetic construct
  VARIANT 56: note = wherein in X is selected from A, G, S, N or T
  source 1..92: note = Portion of SpySwitch variant
DSATHIHFHKHDEDGRELAGATMELRDCSGKTISTWITDGHVKDFYLYPGKYTFVXTAAPDGHHVATPIEFTINEDGQVTVDGEATEGDPHT

SEQ ID NO: 3 - protein, 13 aa, synthetic construct
  source 1..13: note = SpyTag
AHIVMVDAYKPTK

SEQ ID NO: 4 - protein, 14 aa, synthetic construct
  source 1..14: note = SpyTag002
VPTIVMVDAYKRYK

SEQ ID NO: 5 - protein, 16 aa, synthetic construct
  source 1..16: note = SpyTag003
RGVPHIVMVDAYKRYK

SEQ ID NO: 6 - protein, 113 aa, synthetic construct
  source 1..113: note = SpySwitch
VTTLSGLSGEQGPSGDMTTEEDSATHIHFHKHDEDGRELAGATMELRDCSGKTISTWITDGHVKDFYLYPGKYTFVATAAPDGHHVATPIEFTINEDGQVTVDGEATEGDPHT

SEQ ID NO: 7 - protein, 92 aa, synthetic construct
  source 1..92: note = Portion of SpySwitch
DSATHIHFHKHDEDGRELAGATMELRDCSGKTISTWITDGHVKDFYLYPGKYTFVATAAPDGHHVATPIEFTINEDGQVTVDGEATEGDPHT

SEQ ID NO: 8 - DNA, 339 bp, synthetic construct
  source 1..339: mol_type = other DNA; note = DNA encoding SpySwitch
gtaaccaccttatcaggtttatcaggtgagcaaggtccgtccggtgatatgacaactgaagaagatagtgctacccatattcacttccataaacatgatgaggacggccgtgagttagctggtgcaactatggagttgcgtgattgctctggtaaaactattagtacatggattacagatggacatgtgaaggatttctacctgtatccaggaaaatatacatttgtcgcgaccgcagcaccagacggtcatcacgtagcaactccaattgaatttacaattaatgaggacggtcaggttactgtagatggtgaagcaactgaaggtgaccctcatact

SEQ ID NO: 9 - DNA, 276 bp, synthetic construct
  source 1..276: mol_type = other DNA; note = DNA encoding portion of SpySwitch
gatagtgctacccatattcacttccataaacatgatgaggacggccgtgagttagctggtgcaactatggagttgcgtgattgctctggtaaaactattagtacatggattacagatggacatgtgaaggatttctacctgtatccaggaaaatatacatttgtcgcgaccgcagcaccagacggtcatcacgtagcaactccaattgaatttacaattaatgaggacggtcaggttactgtagatggtgaagcaactgaaggtgaccctcatact

SEQ ID NO: 10 - protein, 113 aa, synthetic construct
  source 1..113: note = SpyDock2.0
VTTLSGLSGEQGPSGDMTTEEDSATHIKFHKRDEDGRELAGATMELRDCSGKTISTWISDGHVKDFYLYPGKYTFVATAAPDGHHVATPIEFTVNEDGQVTVDGEATEGDAHT

SEQ ID NO: 11 - protein, 113 aa, synthetic construct
  source 1..113: note = SpyCatcher
VDTLSGLSSEQGQSGDMTIEEDSATHIKFSKRDEDGKELAGATMELRDSSGKTISTWISDGQVKDFYLYPGKYTFVETAAPDGYEVATAITFTVNEQGQVTVNGKATKGDAHI

SEQ ID NO: 12 - protein, 113 aa, synthetic construct
  source 1..113: note = SpyCatcher002
VTTLSGLSGEQGPSGDMTTEEDSATHIKFSKRDEDGRELAGATMELRDSSGKTISTWISDGHVKDFYLYPGKYTFVETAAPDGYEVATAITFTVNEQGQVTVNGEATKGDAHT

SEQ ID NO: 13 - protein, 113 aa, synthetic construct
  source 1..113: note = SpyCatcher003
VTTLSGLSGEQGPSGDMTTEEDSATHIKFSKRDEDGRELAGATMELRDSSGKTISTWISDGHVKDFYLYPGKYTFVETAAPDGYEVATPIEFTVNEDGQVTVDGEATEGDAHT

SEQ ID NO: 14 - protein, 7 aa, synthetic construct
  source 1..7: note = TEV recognition site
ENLYFQG

SEQ ID NO: 15 - protein, 113 aa, synthetic construct
  source 1..113: note = SpyDock
VTTLSGLSGEQGPSGDMTTEEDSATHIKFSKRDEDGRELAGATMELRDCSGKTISTWISDGHVKDFYLYPGKYTFVATAAPDGYEVATPITFTVNEDGQVTVNGEATEGDAHT

SEQ ID NO: 16 - protein, 136 aa, synthetic construct
  source 1..136: note = SpySwitch + His-tag and linkers
MSYYHHHHHHGSGGSGAMVTTLSGLSGEQGPSGDMTTEEDSATHIHFHKHDEDGRELAGATMELRDCSGKTISTWITDGHVKDFYLYPGKYTFVATAAPDGHHVATPIEFTINEDGQVTVDGEATEGDPHTGSSGS

SEQ ID NO: 17 - DNA, 414 bp, synthetic construct
  source 1..414: mol_type = other DNA; note = DNA encoding SpySwitch + His-tag and linkers
atgtcgtactaccatcaccatcaccatcacggtagcggcggtagcggcgccatggtaaccaccttatcaggtttatcaggtgagcaaggtccgtccggtgatatgacaactgaagaagatagtgctacccatattcacttccataaacatgatgaggacggccgtgagttagctggtgcaactatggagttgcgtgattgctctggtaaaactattagtacatggattacagatggacatgtgaaggatttctacctgtatccaggaaaatatacatttgtcgcgaccgcagcaccagacggtcatcacgtagcaactccaattgaatttacaattaatgaggacggtcaggttactgtagatggtgaagcaactgaaggtgaccctcatactggatccagtggtagctaataa

SEQ ID NO: 18 - protein, 6 aa, synthetic construct
  source 1..6: note = Spacer sequence
GSGGSG

SEQ ID NO: 19 - protein, 5 aa, synthetic construct
  source 1..5: note = Spacer sequence
GSSGS